European Patent Application EP 4 242 298 A2, published September 13, 2023. Title: NANOPARTICLE FORMULATIONS. Applicant: TAIGA BIOTECHNOLOGIES, INC. Application EP. The sequence listing filed with the application follows.

SEQUENCE LISTING (44 sequences)

SEQ ID NO: 1 - protein, 476 aa, synthetic construct
  REGION 1..476: note = Description of Artificial Sequence: Synthetic polypeptide
MRKKRRQRRRPLNVSFTNRNYDLDYDSVQPYFYCDEEENFYQQQQQSELQPPAPSEDIWKKFELLPTPPLSPSRRSGLCSPSYVAVTPFSLRGDNDGGGGSFSTADQLEMVTELLGGDMVNQSFICDPDDETFIKNIIIQDCMWSGFSAAAKLVSEKLASYQAARKDSGSPNPARGHSVCSTSSLYLQDLSAAASECIDPSVVFPYPLNDSSSPKSCASQDSSAFSPSSDSLLSSTESSPQGSPEPLVLHEETPPTTSSDSEEEQEDEEEIDVVSVEKRQAPGKRSESGSPSAGGHSKPPHSPLVLKRCHVSTHQHNYAAPPSTRKDYPAAKRVKLDSVRVLRQISNNRKCTSPRSSDTEENVKRRTHNVLERQRRNELKRSFFALRDQIPELENNEKAPKVVILKKATAYILSVQAEEQKLISEEDLLRKRREQLKHKLEQLRKGELNSKLEGKPIPNPLLGLDSTRTGHHHHHH

SEQ ID NO: 2 - protein, 454 aa, Homo sapiens
MDFFRVVENQQPPATMPLNVSFTNRNYDLDYDSVQPYFYCDEEENFYQQQQQSELQPPAPSEDIWKKFELLPTPPLSPSRRSGLCSPSYVAVTPFSLRGDNDGGGGSFSTADQLEMVTELLGGDMVNQSFICDPDDETFIKNIIIQDCMWSGFSAAAKLVSEKLASYQAARKDSGSPNPARGHSVCSTSSLYLQDLSAAASECIDPSVVFPYPLNDSSSPKSCASQDSSAFSPSSDSLLSSTESSPQGSPEPLVLHEETPPTTSSDSEEEQEDEEEIDVVSVEKRQAPGKRSESGSPSAGGHSKPPHSPLVLKRCHVSTHQHNYAAPPSTRKDYPAAKRVKLDSVRVLRQISNNRKCTSPRSSDTEENVKRRTHNVLERQRRNELKRSFFALRDQIPELENNEKAPKVVILKKATAYILSVQAEEQKLISEEDLLRKRREQLKHKLEQLRNSCA

SEQ ID NO: 3 - protein, 459 aa, synthetic construct
  REGION 1..459: note = Description of Artificial Sequence: Synthetic polypeptide
MDFFRVVENQQPPATMPLNVSFTNRNYDLDYDSVQPYFYCDEEENFYQQQQQSELQPPAPSEDIWKKFELLPTPPLSPSRRSGLCSPSYVAVTPFSLRGDNDGGGGSFSTADQLEMVTELLGGDMVNQSFICDPDDETFIKNIIIQDCMWSGFSAAAKLVSEKLASYQAARKDSGSPNPARGHSVCSTSSLYLQDLSAAASECIDPSVVFPYPLNDSSSPKSCASQDSSAFSPSSDSLLSSTESSPQGSPEPLVLHEETPPTTSSDSEEEQEDEEEIDVVSVEKRQAPGKRSESGSPSAGGHSKPPHSPLVLKRCHVSTHQHNYAAPPSTRKDYPAAKRVKLDSVRVLRQISNNRKCTSPRSSDTEENVKRRTHNVLERQRRNELKRSFFALRDQIPELENNEKAPKVVILKKATAYILSVQAEEQKLISEEDLLRKRREQLKHKLEQLRKGELNSKLE

SEQ ID NO: 4 - protein, 434 aa, synthetic construct
  REGION 1..434: note = Description of Artificial Sequence: Synthetic polypeptide
PLNVSFTNRNYDLDYDSVQPYFYCDEEENFYQQQQQSELQPPAPSEDIWKKFELLPTPPLSPSRRSGLCSPSYVAVTPFSLRGDNDGGGGSFSTADQLEMVTELLGGDMVNQSFICDPDDETFIKNIIIQDCMWSGFSAAAKLVSEKLASYQAARKDSGSPNPARGHSVCSTSSLYLQDLSAAASECIDPSVVFPYPLNDSSSPKSCASQDSSAFSPSSDSLLSSTESSPQGSPEPLVLHEETPPTTSSDSEEEQEDEEEIDVVSVEKRQAPGKRSESGSPSAGGHSKPPHSPLVLKRCHVSTHQHNYAAPPSTRKDYPAAKRVKLDSVRVLRQISNNRKCTSPRSSDTEENVKRRTHNVLERQRRNELKRSFFALRDQIPELENNEKAPKVVILKKATAYILSVQAEEQKLISEEDLLRKRREQLKHKLEQLR

SEQ ID NO: 5 - protein, 67 aa, Homo sapiens
ELKRSFFALRDQIPELENNEKAPKVVILKKATAYILSVQAEEQKLISEEDLLRKRREQLKHKLEQLR

SEQ ID NO: 6 - protein, 14 aa, unidentified
  REGION 1..14: note = Description of Unknown: E-box DNA binding domain sequence
KRRTHNVLERQRRN

SEQ ID NO: 7 - protein, 10 aa, Human immunodeficiency virus 1
MRKKRRQRRR

SEQ ID NO: 8 - protein, 439 aa, Chlorocebus sabaeus
MPLNVSFTNRNYDLDYDSVQPYFYCDEEENFYQQQQQSELQPPAPSEDIWKKFELLPTPPLSPSRRSGLCSPSYVAVTPFSPRGDNDGGGGSFSTADQLEMVTELLGGDMVNQSFICDPDDETFIKNIIIQDCMWSGFSAAAKLVSEKLASYQAARKDSGSPNPARGHSVCSTSSLYLQDLSAAASECIDPSVVFPYPLNDSSSPKSCASPDSSAFSPSSDSLLSSTESSPQASPEPLVLHEETPPTTSSDSEEEQEDEEEIDVVSVEKRQAPGKRSESGSPSAGGHSKPPHSPLVLKRCHVSTHQHNYAAPPSTRKDYPAAKRVKLDSVRVLRQISNNRKCTSPRSSDTEENVKRRTHNVLERQRRNELKRSFFALRDQIPELENNEKAPKVVILKKATAYILSVQAEEQKLISEKDLLRKRREQLKHKLEQLRNSCA

SEQ ID NO: 9 - protein, 434 aa, synthetic construct
  REGION 1..434: note = Description of Artificial Sequence: Synthetic polypeptide
PLNVSFTNRNYDLDYDSVQPYFYCDEEENFYQQQQQSELQPPAPSEDIWKKFELLPTPPLSPSRRSGLCSPSYVAVTPFSLRGDNDGGGGSFSTADQLEMVTELLGGDMVNQSFICDPDDETFIKNIIIQDCMWSGFSAAAKLVSEKLASYQAARKDSGSPNPARGHSVCSTSSLYLQDLSAAASECIDPSVVFPYPLNDSSSPKSCASQDSSAFSPSSDSLLSSTESSPQASPEPLVLHEETPPTTSSDSEEEQEDEEEIDVVSVEKRQAPGKRSESGSPSAGGHSKPPHSPLVLKRCHVSTHQHNYAAPPSTRKDYPAAKRVKLDSVRVLRQISNNRKCTSPRSSDTEENVKRRTHNVLERQRRNELKRSFFALRDQIPELENNEKAPKVVILKKATAYILSVQAEEQKLISEKDLLRKRREQLKHKLEQLR

SEQ ID NO: 10 - protein, 476 aa, synthetic construct
  REGION 1..476: note = Description of Artificial Sequence: Synthetic polypeptide
MRKKRRQRRRPLNVSFTNRNYDLDYDSVQPYFYCDEEENFYQQQQQSELQPPAPSEDIWKKFELLPTPPLSPSRRSGLCSPSYVAVTPFSLRGDNDGGGGSFSTADQLEMVTELLGGDMVNQSFICDPDDETFIKNIIIQDCMWSGFSAAAKLVSEKLASYQAARKDSGSPNPARGHSVCSTSSLYLQDLSAAASECIDPSVVFPYPLNDSSSPKSCASQDSSAFSPSSDSLLSSTESSPQASPEPLVLHEETPPTTSSDSEEEQEDEEEIDVVSVEKRQAPGKRSESGSPSAGGHSKPPHSPLVLKRCHVSTHQHNYAAPPSTRKDYPAAKRVKLDSVRVLRQISNNRKCTSPRSSDTEENVKRRTHNVLERQRRNELKRSFFALRDQIPELENNEKAPKVVILKKATAYILSVQAEEQKLISEKDLLRKRREQLKHKLEQLRKGELNSKLEGKPIPNPLLGLDSTRTGHHHHHH

SEQ ID NO: 11 - protein, 9 aa, synthetic construct
  REGION 1..9: note = Description of Artificial Sequence: Synthetic peptide
KGELNSKLE

SEQ ID NO: 12 - protein, 22 aa, synthetic construct
  REGION 1..22: note = Description of Artificial Sequence: Synthetic peptide
MRKKRRQRRRPLNVSFTNRNYD

SEQ ID NO: 13 - protein, 4 aa, synthetic construct
  REGION 1..4: note = Description of Artificial Sequence: Synthetic peptide
YDLD

SEQ ID NO: 14 - protein, 4 aa, synthetic construct
  REGION 1..4: note = Description of Artificial Sequence: Synthetic peptide
LDYD

SEQ ID NO: 15 - protein, 11 aa, synthetic construct
  REGION 1..11: note = Description of Artificial Sequence: Synthetic peptide
YDSVQPYFYCD

SEQ ID NO: 16 - protein, 24 aa, synthetic construct
  REGION 1..24: note = Description of Artificial Sequence: Synthetic peptide
CDEEENFYQQQQQSELQPPAPSED

SEQ ID NO: 17 - protein, 39 aa, synthetic construct
  REGION 1..39: note = Description of Artificial Sequence: Synthetic polypeptide
EDIWKKFELLPTPPLSPSRRSGLCSPSYVAVTPFSLRGD

SEQ ID NO: 18 - protein, 4 aa, synthetic construct
  REGION 1..4: note = Description of Artificial Sequence: Synthetic peptide
GDND

SEQ ID NO: 19 - protein, 12 aa, synthetic construct
  REGION 1..12: note = Description of Artificial Sequence: Synthetic peptide
NDGGGGSFSTAD

SEQ ID NO: 20 - protein, 14 aa, synthetic construct
  REGION 1..14: note = Description of Artificial Sequence: Synthetic peptide
ADQLEMVTELLGGD

SEQ ID NO: 21 - protein, 11 aa, synthetic construct
  REGION 1..11: note = Description of Artificial Sequence: Synthetic peptide
GDMVNQSFICD

SEQ ID NO: 22 - protein, 4 aa, synthetic construct
  REGION 1..4: note = Description of Artificial Sequence: Synthetic peptide
CDPD

SEQ ID NO: 23 - skipped

SEQ ID NO: 24 - protein, 13 aa, synthetic construct
  REGION 1..13: note = Description of Artificial Sequence: Synthetic peptide
DDETFIKNIIIQD

SEQ ID NO: 25 - protein, 28 aa, synthetic construct
  REGION 1..28: note = Description of Artificial Sequence: Synthetic peptide
QDCMWSGFSAAAKLVSEKLASYQAARKD

SEQ ID NO: 26 - protein, 24 aa, synthetic construct
  REGION 1..24: note = Description of Artificial Sequence: Synthetic peptide
KDSGSPNPARGHSVCSTSSLYLQD

SEQ ID NO: 27 - protein, 12 aa, synthetic construct
  REGION 1..12: note = Description of Artificial Sequence: Synthetic peptide
QDLSAAASECID

SEQ ID NO: 28 - protein, 13 aa, synthetic construct
  REGION 1..13: note = Description of Artificial Sequence: Synthetic peptide
IDPSVVFPYPLND

SEQ ID NO: 29 - protein, 13 aa, synthetic construct
  REGION 1..13: note = Description of Artificial Sequence: Synthetic peptide
NDSSSPKSCASQD

SEQ ID NO: 30 - protein, 11 aa, synthetic construct
  REGION 1..11: note = Description of Artificial Sequence: Synthetic peptide
QDSSAFSPSSD

SEQ ID NO: 31 - protein, 32 aa, synthetic construct
  REGION 1..32: note = Description of Artificial Sequence: Synthetic polypeptide
SDSLLSSTESSPQGSPEPLVLHEETPPTTSSD

SEQ ID NO: 32 - protein, 9 aa, synthetic construct
  REGION 1..9: note = Description of Artificial Sequence: Synthetic peptide
SDSEEEQED

SEQ ID NO: 33 - protein, 7 aa, synthetic construct
  REGION 1..7: note = Description of Artificial Sequence: Synthetic peptide
EDEEEID

SEQ ID NO: 34 - protein, 57 aa, synthetic construct
  REGION 1..57: note = Description of Artificial Sequence: Synthetic polypeptide
IDVVSVEKRQAPGKRSESGSPSAGGHSKPPHSPLVLKRCHVSTHQHNYAAPPSTRKD

SEQ ID NO: 35 - protein, 12 aa, synthetic construct
  REGION 1..12: note = Description of Artificial Sequence: Synthetic peptide
KDYPAAKRVKLD

SEQ ID NO: 36 - protein, 23 aa, synthetic construct
  REGION 1..23: note = Description of Artificial Sequence: Synthetic peptide
LDSVRVLRQISNNRKCTSPRSSD

SEQ ID NO: 37 - protein, 32 aa, synthetic construct
  REGION 1..32: note = Description of Artificial Sequence: Synthetic polypeptide
SDTEENVKRRTHNVLERQRRNELKRSFFALRD

SEQ ID NO: 38 - protein, 41 aa, synthetic construct
  REGION 1..41: note = Description of Artificial Sequence: Synthetic polypeptide
RDQIPELENNEKAPKVVILKKATAYILSVQAEEQKLISEED

SEQ ID NO: 39 - protein, 40 aa, synthetic construct
  REGION 1..40: note = Description of Artificial Sequence: Synthetic polypeptide
EDLLRKRREQLKHKLEQLRKGELNSKLEGKPIPNPLLGLD

SEQ ID NO: 40 - protein, 13 aa, synthetic construct
  REGION 1..13: note = Description of Artificial Sequence: Synthetic peptide
LDSTRTGHHHHHH

SEQ ID NO: 41 - protein, 6 aa, synthetic construct
  REGION 1..6: note = Description of Artificial Sequence: Synthetic 6xHis tag
HHHHHH

SEQ ID NO: 42 - protein, 14 aa, synthetic construct
  REGION 1..14: note = Description of Artificial Sequence: Synthetic peptide
GKPIPNPLLGLDST

SEQ ID NO: 43 - protein, 9 aa, synthetic construct
  REGION 1..9: note = Description of Artificial Sequence: Synthetic peptide
IPNPLLGLD

SEQ ID NO: 44 - protein, 9 aa, Human immunodeficiency virus 1
RKKRRQRRR